European Patent Specification EP 3 903 820 B1, published May 7, 2025. Title: METHODS FOR TREATING GI SYNDROME AND GRAFT VERSUS HOST DISEASE. Applicant: SLOAN KETTERING INSTITUTE FOR CANCER. Application PCT/US2013/042941. The sequence listing filed with the application follows.

SEQUENCE LISTING (8 sequences)

SEQ ID NO: 1 - protein, 115 aa, Mouse sp.
  misc_feature: Mouse 2A2 Variable Heavy Chain (VH)
EVQLQQSGTVLARPGASVKMSCKASGYTFTNYWMHWVKQRPVQGLEWIGAIYPGDSDTSYNQKFKGKAKLTAVTSTSTAFMELSSLTNEDSAVYYCTGLYYGYDWGQGTTLTVSS

SEQ ID NO: 2 - protein, 129 aa, Homo sapiens
  misc_feature: Human germline 2A2 Variable Heavy Chain of the 2A2 antibody
QVQLVQSGAEVKKPGASVKVSCKASGYTFTSYYMHWVRQAPGQGLEWMGIINPSGGSTSYAQKFQGRVTMTRDTSTSTVYMELSSLRVTMTRDTSTSTVYMELSSLRSEDTAVYYCARWGQGTTVTVSS

SEQ ID NO: 3 - protein, 112 aa, Mouse sp.
  misc_feature: Mouse 2A2 Variable Light Chain (VL)
DVLMTQTPLTLSVTIGQPASISCKSSQSLIDSDGKTFLNWLLQRPGQSPKRLIYLVSKLDSGVPDRFTGSGSGTDFTLKISRVEAEDLGLYYCWQGTHFPYTFGGGTKLEIK

SEQ ID NO: 4 - protein, 112 aa, Homo sapiens
  misc_feature: Human germline 2A2 Variable Light (VL)
DVVMTQSPLSLPVTLGQPASISCRSSQSLVYSDGNTYLNWFQQRPGQSPRRLIYKVSNWDSGVPDRFSGSGSGTDFTLKISRVEAEDVGVYYCMQGTHWPTFGQGTKLEIKR

SEQ ID NO: 5 - DNA, 1395 bp, Artificial Sequence
  HUMANIZED 2A2 HEAVY CHAIN DNA SEQUENCE
atggactggacctggagggtcttctgcttgctggctgtagctccaggtgctcactcccaggtgcagcttgtgcagtctggggctgaggtgaaaaagcctggggcttcagtgaaggtgtcctgcaaggcttctggctacacctttaccaactactggatgcactgggtaagacaggcgcctggacagggtctggaatggatgggcgctatttatcctggagatagtgatactagctacaaccagaagttcaagggccgggtcacaatgactcgagacacatccaccagcactgtctacatggagctcagcagcctgagaagtgaggacactgcggtctattactgtgcacgcctttactacggctacgactggggccaaggcaccactgtcacagtctcctcagccagcacgaagggcccatcggtcttccccctggcaccctcctccaagagcacctctgggggcacagcggccctgggctgcctggtcaaggactacttccccgaaccggtgacggtgtcgtggaactcaggcgccctgaccagcggcgtgcacaccttcccggctgtcctacagtcctcaggactctactccctcagcagcgtggtgaccgtgccctccagcagcttgggcacccagacctacatctgcaacgtgaatcacaagcccagcaacaccaaggtggacaagaaagttgagcccaaatcttgtgacaaaactcacacatgcccaccgtgcccagcacctgaactcctggggggaccgtcagtcttcctcttccccccaaaacccaaggacaccctcatgatctcccggacccctgaggtcacatgcgtggtggtggacgtgagccacgaagaccctgaggtcaagttcaactggtacgtggacggcgtggaggtgcataatgccaagacaaagccgcgggaggagcagtacaacagcacgtaccgtgtggtcagcgtcctcaccgtcctgcaccaggactggctgaatggcaaggagtacaagtgcaaggtctccaacaaagccctcccagcccccatcgagaaaaccatctccaaagccaaagggcagccccgagaaccacaggtgtacaccctgcccccatcccgggatgagctgaccaagaaccaggtcagcctgacctgcctggtcaaaggcttctatcccagcgacatcgccgtggagtgggagagcaatgggcagccggagaacaactacaagaccacgcctcccgtgctggactccgacggctccttcttcctctacagcaagctcaccgtggacaagagcaggtggcagcaggggaacgtcttctcatgctccgtgatgcatgaggctctgcacaaccactacacgcagaagagcctctccctgtccccgggtaaatga

SEQ ID NO: 6 - protein, 463 aa, Artificial Sequence
  AMINO ACID SEQUENCE OF HUMANIZED 2A2 HEAVY CHAIN
MDWTWRVFCLLAVAPGAHSQVQLVQSGAEVKKPGASVKVSCKASGYTFTNYWMHWVRQAPGQGLEWMGAIYPGDSDTSYNQKFKGRVTMTRDTSTSTVYMELSSLRSEDTAVYYCARLYYGYDWGQGTTVTVSSASTKGPSVFPLAPSSKSTSGGTAALGCLVKDYFPEPVTVSWNSGALTSGVHTFPAVLQSSGLYSLSSVVTVPSSSLGTQTYICNVNHKPSNTKVDKKVEPKSCDKTHTCPPCPAPELLGGPSVFLFPPKPKDTLMISRTPEVTCVVVDVSHEDPEVKFNWYVDGVEVHNAKTKPREEQYNSTYRVVSVLTVLHQDWLNGKEYKCKVSNKALPAPIEKTISKAKGQPREPQVYTLPPSRDELTKNQVSLTCLVKGFYPSDIAVEWESNGQPENNYKTTPPVLDSDGSFFLYSKLTVDKSRWQQGNVFSCSVMHEALHNHYTQKSLSLSPG

SEQ ID NO: 7 - DNA, 720 bp, Artificial Sequence
  HUMANIZED 2A2 LIGHT CHAIN DNA SEQUENCE
atgaggctccctgctcagctcctggggctgctaatgctctgggtcccaggatccagtggggatgttgtgatgacccaatctccactctctttgccggttacccttggacaaccagcctccatctcttgcaagtcaagtcagagcctcatagatagtgatggaaagacatttttgaattggttccaacagaggccaggccagtctccaaggcgcctaatctatctggtgtctaaactggactctggagtccctgacaggttctctggcagtggatcagggacagatttcactctgaaaatcagcagagtggaggctgaggatgtgggagtttattattgctggcaaggtacacattttccgtacacgttcggacaggggaccaagctggaaataaaacggacggtggctgcaccatctgtcttcatcttcccgccatctgatgagcagttgaaatctggaactgcctctgttgtgtgcctgctgaataacttctatcccagagaggccaaagtacagtggaaggtggataacgccctccaatcgggtaactcccaggagagtgtcacagagcaggacagcaaggacagcacctacagcctcagcagcaccctgacgctgagcaaagcagactacgagaaacacaaagtctacgcctgcgaagtcacccatcagggcctgagttcgcccgtcacaaagagcttcaacaggggagagtgttaa

SEQ ID NO: 8 - protein, 239 aa, Artificial Sequence
  AMINO ACID SEQUENCE OF HUMANIZED 2A2 LIGHT CHAIN
MRLPAQLLGLLMLWVPGSSGDVVMTQSPLSLPVTLGQPASISCKSSQSLIDSDGKTFLNWFQQRPGQSPRRLIYLVSKLDSGVPDRFSGSGSGTDFTLKISRVEAEDVGVYYCWQGTHFPYTFGQGTKLEIKRTVAAPSVFIFPPSDEQLKSGTASVVCLLNNFYPREAKVQWKVDNALQSGNSQESVTEQDSKDSTYSLSSTLTLSKADYEKHKVYACEVTHQGLSSPVTKSFNRGEC